European Patent Specification EP 3 472 188 B1, published August 5, 2026. Title: Nematode Resistance. Applicant: KeyGene N.V. The sequence listing filed with the application follows.

SEQUENCE LISTING (15 sequences)

SEQ ID NO: 1 - protein, 511 aa, Solanaceae
  misc_feature (21)..(21): Xaa can be any naturally occurring amino acid
  misc_feature (191)..(191): Xaa can be any naturally occurring amino acid
  misc_feature (265)..(265): Xaa can be any naturally occurring amino acid
  misc_feature (287)..(287): Xaa can be any naturally occurring amino acid
  misc_feature (335)..(335): Xaa can be any naturally occurring amino acid
  misc_feature (346)..(346): Xaa can be any naturally occurring amino acid
  misc_feature (349)..(349): Xaa can be any naturally occurring amino acid
MDDENESSKSAGLKNSNLEEXEDKISNKIENSSVHNDDNGDDRVIDGSSGAESLRESKTEALISETLAHPNAESSVQIEIDGQSEFDSEFSPSYQLSEVPVEYELPSFGFSEKIKDRISVTKPGTLNAQARTEHQRRVPDAASSLELSSLSVAQSISSVPSATLAERRSAAAVNCSTGEVVKQSSDAQVLXLVPVLKRPTRDGYNWRKYGQKQVKSPQGSRSYYRCTHSECCAKKIECSDHTNRVMEIIYRTQHNHDPPPRVNCXRESKSAVLSSPTNGKSIIAHPXRNSIETVVSSLKENLQESLPIAETANQDSGGSDTDTEITIREEHRDEXGQKKRSRKSDXSCXESVSKPGKKPKLVVHAACDVGISSDGYRWRKYGQKMVKGNPHPRNYYRCTSAGCPVRKHIERVVDTTSALTITYKGVHDHDMPVPKKRHGPPSAPLIAATAPASVTNMHANKPEPLQHQKSTTQWSVDKEGELTGEKLDVGGEKAMESARTLLSIGFEIKPC

SEQ ID NO: 2 - protein, 467 aa, Brassicaceae
  misc_feature (5)..(5): Xaa can be any naturally occurring amino acid
  misc_feature (77)..(77): Xaa can be any naturally occurring amino acid
  misc_feature (92)..(92): Xaa can be any naturally occurring amino acid
  misc_feature (104)..(104): Xaa can be any naturally occurring amino acid
  misc_feature (109)..(109): Xaa can be any naturally occurring amino acid
  misc_feature (112)..(112): Xaa can be any naturally occurring amino acid
  misc_feature (124)..(124): Xaa can be any naturally occurring amino acid
  misc_feature (132)..(133): Xaa can be any naturally occurring amino acid
  misc_feature (246)..(246): Xaa can be any naturally occurring amino acid
  misc_feature (265)..(265): Xaa can be any naturally occurring amino acid
  misc_feature (318)..(318): Xaa can be any naturally occurring amino acid
  misc_feature (320)..(320): Xaa can be any naturally occurring amino acid
  misc_feature (375)..(375): Xaa can be any naturally occurring amino acid
MEDKXSDEADVYAAAETEKSEKVEPEKELCDGLSQLRDEEESLGADMEDLHDEPVRETLAKDQVEGVRENSSVEPNXEDVKEVKETDSGKEXVVSAIVPVDEVXVENRXVEXSPCLTASSDPSXVEPSLSSXXSAAQGLSLVSVPTKQEQRSDSRVVNNLSVSPVLRTPARDGYNWRKYGQKQVKSPKGSRSYYRCTYSECCAKKIECSNDSGNVIEIVNKGLHSHEPPRKNSFSPREIRAASAIXPVSEDNTVVEEIVPSGSDXSASTKENICQSLTIVERKRHCENEAVEEPEPKRRLKKDNSQSSDSVSKPGKKXKXVVHAAGDVGISGDGYRWRKYGQKMVKGNPNPRNYYRCTSAGCPVRKHIETAVENXTAVIITYKGVHNHDMPVPKKRHGPPSSMLVAAAAPTSMRTRLDDQVNIPTSSQCSVGRESEKQSSEAVDVGGEKVMESARTLLSIGFEIKQC

SEQ ID NO: 3 - protein, 487 aa, Cucurbitaceae
  misc_feature (19)..(20): Xaa can be any naturally occurring amino acid
  misc_feature (23)..(23): Xaa can be any naturally occurring amino acid
  misc_feature (35)..(35): Xaa can be any naturally occurring amino acid
  misc_feature (38)..(38): Xaa can be any naturally occurring amino acid
  misc_feature (40)..(40): Xaa can be any naturally occurring amino acid
  misc_feature (52)..(52): Xaa can be any naturally occurring amino acid
  misc_feature (66)..(66): Xaa can be any naturally occurring amino acid
  misc_feature (69)..(69): Xaa can be any naturally occurring amino acid
  misc_feature (73)..(73): Xaa can be any naturally occurring amino acid
  misc_feature (104)..(104): Xaa can be any naturally occurring amino acid
  misc_feature (143)..(143): Xaa can be any naturally occurring amino acid
  misc_feature (147)..(147): Xaa can be any naturally occurring amino acid
  misc_feature (237)..(237): Xaa can be any naturally occurring amino acid
  misc_feature (300)..(300): Xaa can be any naturally occurring amino acid
  misc_feature (308)..(308): Xaa can be any naturally occurring amino acid
  misc_feature (310)..(310): Xaa can be any naturally occurring amino acid
  misc_feature (433)..(433): Xaa can be any naturally occurring amino acid
MEDSDDESEVELEGEGGGXXSEXKPTELRTGSSVXEAXVXGSLSETLTVASXNQSSENGRSDGLPXNSXAQSXEGAELKQAPSSHSEPLAVEATQTDKVQEQNXLQLTVFKGPDSEQSPTSVTQSISSSASPNLSEHKLSPKXVQKXCKPEPSQKNFFNHKTPSSVPNARTPASDGYNWRKYGQKQVKSPKGSRSYYKCTYSECFAKKIECCDDSGQTTEIVYKSQHSHDPPRKISXPKESKLVPYVEPVVKKIIAEHSRRVINDSDPPTSSKEPLRETAIVVFERKRQYSNDSNGNDEXKIKDENDXEXETKQKVKKSSAGNSGTPLKPGKKPKFVVHAAGDVGISGDGYRWRKYGQKMVKGNPHPRNYYRCTSAGCPVRKHIESAVENPNAVIITYKGVHDHDTPVPKKRHGPPSALLVAAAAPASMSSNXQPKKTDVVESQISSTQWSVDAEGELTGEALELGGEKAMESARTLLSIGFEIKPC

SEQ ID NO: 4 - protein, 503 aa, Fabaceae
  misc_feature (14)..(17): Xaa can be any naturally occurring amino acid
  misc_feature (21)..(21): Xaa can be any naturally occurring amino acid
  misc_feature (29)..(29): Xaa can be any naturally occurring amino acid
  misc_feature (33)..(33): Xaa can be any naturally occurring amino acid
  misc_feature (45)..(45): Xaa can be any naturally occurring amino acid
  misc_feature (90)..(90): Xaa can be any naturally occurring amino acid
  misc_feature (108)..(108): Xaa can be any naturally occurring amino acid
  misc_feature (165)..(165): Xaa can be any naturally occurring amino acid
  misc_feature (275)..(275): Xaa can be any naturally occurring amino acid
  misc_feature (284)..(284): Xaa can be any naturally occurring amino acid
  misc_feature (301)..(301): Xaa can be any naturally occurring amino acid
  misc_feature (306)..(306): Xaa can be any naturally occurring amino acid
MAERGSPQLLPEPXXXXNDSXQKPKAAEXTERXTESPSAAESQRXELRSSDEPRTESNLETLGAASSVTLAVQHHRSDDLQGSSAAPNSXGKAESKETVGPPEKEIIXRGAAQPLPTQTENRLQVSVCSTPLSELSPTSVTQSLSSVSSPTVPKQKMSTPKVNNXHVPEVDKKNPSGGKTLSAVSVARTSASDGYNWRKYGQKQVKSPTGSRSYYRCTHSDCCAKKIECCDHSGHVIEIVYKSEHSHDPPRKTNSIRENKFLSSSEPIVENSVPXQPVRVLKDXDPSISSKESLQEAPCSXDKKRXNSSNISGNGKVILKEEHVNEPEPKKRMKKGDLTDMDSPVKPGKKPKFVVHAAGDVGISGDGYRWRKYGQKMVKGNPHPRNYYRCTSAGCPVRKHIETAVDNSDAVIITYKGVHDHDMPVPKKRHGPPSAPLVAAAAPASMNSLQVKKPDSPQNKKISTQWSVDTEGELTGEALELGGEKAMESARTLLSIGFEIKPC

SEQ ID NO: 5 - protein, 506 aa, Rosaceae
  misc_feature (4)..(4): Xaa can be any naturally occurring amino acid
  misc_feature (8)..(8): Xaa can be any naturally occurring amino acid
  misc_feature (12)..(13): Xaa can be any naturally occurring amino acid
  misc_feature (17)..(17): Xaa can be any naturally occurring amino acid
  misc_feature (19)..(21): Xaa can be any naturally occurring amino acid
  misc_feature (26)..(27): Xaa can be any naturally occurring amino acid
  misc_feature (33)..(33): Xaa can be any naturally occurring amino acid
  misc_feature (35)..(35): Xaa can be any naturally occurring amino acid
  misc_feature (37)..(39): Xaa can be any naturally occurring amino acid
  misc_feature (44)..(44): Xaa can be any naturally occurring amino acid
  misc_feature (46)..(46): Xaa can be any naturally occurring amino acid
  misc_feature (50)..(51): Xaa can be any naturally occurring amino acid
  misc_feature (53)..(54): Xaa can be any naturally occurring amino acid
  misc_feature (56)..(56): Xaa can be any naturally occurring amino acid
  misc_feature (70)..(70): Xaa can be any naturally occurring amino acid
  misc_feature (78)..(78): Xaa can be any naturally occurring amino acid
  misc_feature (81)..(81): Xaa can be any naturally occurring amino acid
  misc_feature (84)..(84): Xaa can be any naturally occurring amino acid
  misc_feature (86)..(86): Xaa can be any naturally occurring amino acid
  misc_feature (94)..(94): Xaa can be any naturally occurring amino acid
  misc_feature (101)..(101): Xaa can be any naturally occurring amino acid
  misc_feature (112)..(112): Xaa can be any naturally occurring amino acid
  misc_feature (117)..(117): Xaa can be any naturally occurring amino acid
  misc_feature (122)..(123): Xaa can be any naturally occurring amino acid
  misc_feature (155)..(155): Xaa can be any naturally occurring amino acid
  misc_feature (159)..(159): Xaa can be any naturally occurring amino acid
  misc_feature (161)..(161): Xaa can be any naturally occurring amino acid
  misc_feature (275)..(275): Xaa can be any naturally occurring amino acid
  misc_feature (336)..(336): Xaa can be any naturally occurring amino acid
  misc_feature (345)..(345): Xaa can be any naturally occurring amino acid
  misc_feature (408)..(408): Xaa can be any naturally occurring amino acid
  misc_feature (461)..(461): Xaa can be any naturally occurring amino acid
MAEXHESXDALXXEKLXPXXXEQEEXXEGDEDXDXEXXXRLGEXQXGELXXSXXEXRETQLETLAVPSTXELSENDQXAGXQVXSXSQSIDGAXLQEQLGXSHQEILASVTXQDSQXQTQSXXQLQLTVYPTPLSELSPTSVTQSISSAPSPILXEQRXPXEKVNTLCTPEVDKQNSSDHKFISSVPLVKTSASDGYNWRKYGQKQVKSPQGSRSYYRCTYSECYAKKIECCDHSGHVTEIVYKSQHTHDPPRKSNCTKESKLALSAECVRNSVXEHPCRTVNDSEVSTSSKEPIQETPSVPERKRQSPSDSDGNGDVKIKEEHGDGDEPEPKRRXKKSNSEYSXSLLKPGKKPKFVVHAAGDVGISGDGYRWRKYGQKMVKGNPHPRNYYRCTSAGCPVRKHIETAXDNTSAVIITYKGIHDHDMPVPKKRHGPPSAPLVAAAAPASMNNLHIKKTDTHXNQISSTQWSVDTGGELTGEALDLGGEKAMESARTLLSIGFEIKPC

SEQ ID NO: 6 - protein, 558 aa, Poaceae
  misc_feature (9)..(9): Xaa can be any naturally occurring amino acid
  misc_feature (12)..(12): Xaa can be any naturally occurring amino acid
  misc_feature (36)..(36): Xaa can be any naturally occurring amino acid
  misc_feature (38)..(38): Xaa can be any naturally occurring amino acid
  misc_feature (43)..(43): Xaa can be any naturally occurring amino acid
  misc_feature (45)..(46): Xaa can be any naturally occurring amino acid
  misc_feature (54)..(55): Xaa can be any naturally occurring amino acid
  misc_feature (62)..(62): Xaa can be any naturally occurring amino acid
  misc_feature (66)..(66): Xaa can be any naturally occurring amino acid
  misc_feature (69)..(69): Xaa can be any naturally occurring amino acid
  misc_feature (74)..(74): Xaa can be any naturally occurring amino acid
  misc_feature (82)..(82): Xaa can be any naturally occurring amino acid
  misc_feature (90)..(90): Xaa can be any naturally occurring amino acid
  misc_feature (97)..(97): Xaa can be any naturally occurring amino acid
  misc_feature (99)..(99): Xaa can be any naturally occurring amino acid
  misc_feature (103)..(105): Xaa can be any naturally occurring amino acid
  misc_feature (107)..(107): Xaa can be any naturally occurring amino acid
  misc_feature (113)..(113): Xaa can be any naturally occurring amino acid
  misc_feature (118)..(118): Xaa can be any naturally occurring amino acid
  misc_feature (126)..(126): Xaa can be any naturally occurring amino acid
  misc_feature (193)..(193): Xaa can be any naturally occurring amino acid
  misc_feature (196)..(196): Xaa can be any naturally occurring amino acid
  misc_feature (213)..(213): Xaa can be any naturally occurring amino acid
  misc_feature (218)..(218): Xaa can be any naturally occurring amino acid
  misc_feature (224)..(224): Xaa can be any naturally occurring amino acid
  misc_feature (226)..(226): Xaa can be any naturally occurring amino acid
  misc_feature (299)..(299): Xaa can be any naturally occurring amino acid
  misc_feature (304)..(304): Xaa can be any naturally occurring amino acid
  misc_feature (313)..(313): Xaa can be any naturally occurring amino acid
  misc_feature (328)..(328): Xaa can be any naturally occurring amino acid
  misc_feature (337)..(337): Xaa can be any naturally occurring amino acid
  misc_feature (342)..(342): Xaa can be any naturally occurring amino acid
  misc_feature (447)..(447): Xaa can be any naturally occurring amino acid
  misc_feature (479)..(479): Xaa can be any naturally occurring amino acid
  misc_feature (485)..(485): Xaa can be any naturally occurring amino acid
  misc_feature (491)..(491): Xaa can be any naturally occurring amino acid
  misc_feature (508)..(509): Xaa can be any naturally occurring amino acid
MADGDPAAXPEXKRPAPEAAEAEAHPPPEPPGAKPXEXEEGEXGXXKEEKVEAXXDMEGKGXEKEXGDXAKEKXEEEDKGKXKEGKGKEXETKEKVXVXAKKXXXAXEKEKGXEKEVXATRRPAGXSAETPILAVPMVAVPCFIAPPGFAGQFAMSHQAALASVTAQAQMQLQSPTTSAYSEGLPSPFPITPXAVXPLQQSPSVTEGNVCRPXAEKSXSSQSKXPXHHVSVNMVGDGFNWRKYGQKQVKSSENSRSYYRCTNSGCLAKKKVEHCPDGRVVEIIYRGTHNHEPPQKTRFXKERVXHITVSSGDXETLRLVNTEIIESSXPPGCKLEPXAVSEXSEQQLFCSSDCEGDAGNKSEDEHPSAEPQPKRRIIETTTPNLTPVLRTVREQKIIVQAGKMSDGYRWRKYGQKIVKGNPNPRSYYRCTHDGCPVRKHVEKAPDDXNNIVVTYEGKHNHDQPFRSSSESVDGPVPMIXPAETTXEQPSTXTSTSDQKPPTSTQKDAXXESDKETTLEFGGEKAVESAQTLLSIKTNPDDMKNSLLKDTSAVVPVQNN

SEQ ID NO: 7 - protein, 511 aa, Solanum
MDDENESSKSTGLKNSNLEEEEDKISNKIENSSVHNDDNGDDRVIDGSSGAESLRESKTEALISETLAHPNAESSVQIEIDGQSEFDSEFSPSYQLSEVPVEYELPSFGFSEKIKDRISVTKPGTLNAQARTEHQRRVPDAASSLELSSLSVAQSISSVPSATLAERRSAAAVNCSTGEVVKQSSDAQVLALVPVLKRPTRDGYNWRKYGQKQVKSPQGSRSYYRCTHSECCAKKIECSDHTNRVMEIIYRTQHNHDPPPRVNCPRESKSALLSSPTNGKSIIAHPSRNSIETVVSSLKENLQESLPIAETANQDSGGSDTDTEITIREEHRDEAGQKKRSRKSDTSCLESVSKPGKKPKLVVHAACDVGISSDGYRWRKYGQKMVKGNPHPRNYYRCTSAGCPVRKHIERVVDTTSALTITYKGVHDHDMPVPKKRHGPPSAPLIAATAPASVTNMHANKPEPLQHQKSTTQWSVDKEGELTGEKLDVGGEKAMESARTLLSIGFEIKPC

SEQ ID NO: 8 - protein, 513 aa, Solanum lycopersicum
MDDENESSKSAGLKNSNLEEEEEDKISNKIENSSVHNDENGDDDRVIDGSSGAESLRESKTGALISETLAHPNAESSVQIEIDGQSEFDSEFSPSYQLSEVPVEYELPSFGFSEKIKDRISVTKPGTLNAQARTEHQRRVPDAASSLELSSLSVAQSISSVPSATLAERRSAAAVNCSTGEVVKQSSDAQVLALVPVLKRPTRDGYNWRKYGQKQVKSPQGSRSYYRCTHSECCAKKIECSDHTNRVMEIIYRTQHNHDPPPRVNCPRESKSALLSSPTNGKSIIAHPRRNSIETVVSPLNENLQESLPIAETANQDSGGSDTDTEITIREEHRDEAGQKKRSRKSDTSCLESVSKPGKKPKLVVHAACDVGISSDGYRWRKYGQKIVKGNPHPRNYYRCTSAGCPVRKHIERVLDTTSALTITYKGVHDHDMPVPKKRHGPPSAPLIAATAPASVTTMHANKPEPLQHQKSTTQWSVDKEGELTGEKLDVGGEKAMESARTLLSIGFEIKPC

SEQ ID NO: 9 - DNA, 1533 bp, Solanum
atggatgacgaaaacgagagctccaaatcaaccggactcaaaaattcaaatctagaagaagaagacaaaatcagcaacaaaatcgaaaattcctccgtacacaacgacgacaacggtgacgatagagtaattgacggtagcagtggagctgagagtttacgagaatcaaagacggaagctttaatttcagaaaccctagctcatcctaatgcagaatcatccgtacaaattgaaattgatggccaatccgaattcgattcagagttttctccctcttatcaactttctgaagtaccagtggaatatgaactgccctcgtttggtttctcggaaaaaatcaaggatagaattagtgttaccaaacctggaactttgaatgctcaagcacgaacagaacatcaacgacgtgttcctgatgcagcatcctcattggagctgtcctctttatctgttgcacagtccatttcatcagtgccaagtgcaactctagcagaaagacgatcagcagcagcagtaaattgtagtacaggagaagtggttaagcagagttctgacgcccaggttctagctcttgtaccagttctaaagagaccaactcgcgatgggtacaattggcggaagtatggtcaaaagcaagttaaaagtcctcaaggttctcgaagttattaccgatgcactcattctgagtgttgtgccaagaagattgagtgctctgatcacactaatcgtgttatggagattatttatagaactcaacacaatcatgatccacccccaagagtaaattgcccaagggaaagcaagtctgcattattgtcttcacctaccaatggcaaaagtataatagctcatccaagtagaaattctattgagaccgtagtatcctccttaaaagaaaatttgcaagaaagtttaccaattgctgagacagcaaatcaggattccggtgggtctgacactgacactgaaatcactattagagaggagcaccgtgacgaggctggacaaaagaagaggtcaaggaaaagtgacacaagttgtttggaatctgtttctaaacctggaaagaaacccaagcttgtggtgcatgctgcttgtgatgtaggaatctcaagtgatggctacagatggcgaaagtatggacaaaaaatggtgaagggaaatccccatccaaggaactactatcgctgtacatcagctggatgtcctgttcgaaagcacattgagagggttgtagataccacaagtgctttaacaataacatacaagggagtacacgatcatgacatgccagtacccaaaaaacgtcatggtccaccgagtgcacctcttattgctgctactgcccctgcttccgtaaccaatatgcatgctaacaaacccgaaccgctacaacatcaaaaatcgaccacacaatggtccgtggacaaagaaggtgagttgactggtgagaaattggatgttggaggagaaaaagcaatggaatcggctcgaactctgttgagtattggatttgaaattaagccttgctaa

SEQ ID NO: 10 - DNA, 6185 bp, Solanum lycopersicum
catttttttcacaaaaacactcactgtgtgttcatcggaatccgccatggatgacgaaaacgagagctccaaatcagccggactcaaaaattcaaatctagaagaagaagaagaagataaaatcagcaacaaaatcgaaaattcctccgtacacaacgacgaaaacggtgacgacgatagagtaattgacggtagcagtggagctgagagtttacgagaatcaaagacgggagctttaatttcagaaaccctagctcatcctaatgcagaatcatccgtacaaattgaaattgatggccaatccgaattcgattcagagttttctccctcttatcaactttctggtactattcaatgccgtttaattcgttcttatgctttttttttgtgtgtgaaattgagtagttcatgtttcattttttatgatcaatttctatacatttgaaccattttttttataatcttgtatccctataacgactctgctaattccacgagatatctgtttcgttccacgagcgtattaagtaacttgtataacatgagaaaaaaaatacaatttatgtgacatgatatcgttttttagtaggttctatagaaaaggacacatttttattatttagtaacaacttaatgttaagatatatcttcacccttagtgagaagtttcaaaagtgttctttttaacatcgcgtaaattgggatgaagaaagtagtagtattttgtctctgctgggaattgaacgtgagattttacgatgcttaacatcttcattgacggctaagccacacacttgggtgctatacttttgaatttctttcctgttttatgtgtatataagcgtagaatgtttagttgttgatcaaaagcacaccgaaagtattatgactagtttccgtattaggtgttcaccttctcattcgaccacctatcaccaattgttcacacacgtgttacgataaatagttgatgattgttcaaatagaaaaggaaaacacctcaactatcatttgtgagtctcatggtcaaggtgtgttttatactaacggacatacacgtgttataatattatccaccgacttgacatttataaaatattagatcgataatgaagattgtgccacgtgtccctgtaagtatagcaaacggtatatgcataccatttatgatagtttggggtatatttgtcctttttcccgtaataaatacttggtggtagtttacgtagaaaaagtgaacaccgaatagttcatatagggaatttgcaaaaagatcttcaggtgcgtttggccattatatctaggaggcaagtccttttgattttatatttttgtgtaagagagattatgatcatgagttctccttatcaaaaagaaataaattatgatcatgagttttatgagtttttaagtagaaaaagggaataagttatacttgaggtgtgttttgacaaatagtcgttaatagatcagataggaaaactgaacatctaatagttcatataggaaacttgcaaaaatgtgatacttcacgtgtattttgaccattatatctggaatgtaagtccttttgagttgtacatgcatgcttaattgtctacgaaaattctgtaattattgtgttgaataatctggcagaagtaccagtggaatatgaactgccctcgtttggtttctcggaaaaaatcaaggtatgcagttcctttcttttgacttggtatttaattttgttatgatagtttatctatttcgagatgtgggagatggttgagtggattcgatgtggtagcatattcttattatattgtagagggagcatacgcactaccctccctggaccccacttatcggattagagtggttatgttgttgtattttaataagttagtttttcaattatcttgttactataatcataggtgtcaatgtatctgaatagtacttactcaaaaaagaaaaaacaagtagtgtatttgaatggtagcacagagatactgaggtaatttacgataggggtggacaacatgcgcaagtagaaaattcaaggtgattgctctgtcactatttggagttttggaccggagagctcgctgcttttttttagtagatatgtacaaggtcgattagaatacagaagttaaattctgctaaagctgaaacttaagtgtcagtataaatcgagccaaaaatttctgcaatataaatcactgaggtttctggagttattgtggtaaacagggtgcatgattatcggttctacaagattctatgcacattccatgttgcatatacaaagttattctgaagatttagaagttcttgtttatcctcatttgcgttttatgaagcatgcgacaaagtagttttgtcttaaaagatcaagttaggtaggagttgaaaatggagtagagtgtcctcgtacacctccttattcatgatggttgatattgggaatcgttagtaggtgatgggcagtctgtagaaatacgttgagctgatgtgtggcatgagcttgagatatcacatacacggtgatgggtattgtaactgtaaatttagacgttttctctgagagagctatataagggtctgatttaaatgtagtaaccccatcatatttatgaagcctctaagaacagtgttttgggaagcgagaagcggaaaaaagcgatgagggttcgctttacagaaggcgatatttagtataaaaataaaattatataaattaactgaatagaggtaatatattcttagattataagaaaatagatagtcaataatacttataagtcataacatataaagcaaaaaaatcaaaaacataattaaatcacaaagaatcaaactcctactcttcaacaagatcctcaaactctttaaaatgcagcaataaaaatataaaaaaacacccagcagtaaccaaaaaaaaaaacaagtagcagatagcagcagcttcgtagagaagaagagaagaagaaaaaaaaacttacagaagcttggcagcaaccaaccaaaaagagtatgaagaagagaagaagaagagaacttgcataaaaaaaagtctgaagaagagaagaagaagagaacttgcataaaaaaaagtctgaagaagagaagaagaagagaacttgcataaaaaaaagtctgaagaagagaagcagtcgcagctgtgagtgaagtcgcgacagatggaaagagtatgtgaagtcgcatatctttctgaaattaaaaaaaaaaacttacaatttttttggaaaaaaaacataaggggcgctttttatgctttatcgcgctttcgtttttctggcgcttctcgcttctacagtagaagcgagcgccttttcaatgtcaccttgcctcaggagctaaaagcgcaagagcatcgcctcactttaagcgcgcttttcacaacactgtctaagacataccgaaaggcttaaatgcacgagataagataactcagagatgatggcctaggctcgaacttgtgacttaaccgggggcgggtggtggtggaaaggggactatatcattactataccagtgtgaggcatagttgttttgtgcattagattttgtttcctaaatgagcaatgaagtgggtgcaaaccttggagaataccagtagagacaaaaaaacactaggtgttttcccatctgtctgagccttagggttatagttatccggtactcatgttggtggataatactcaagtagcaggtaccgcttgaggaatcatcatgatcctttagttttggataaattgaaagcagatgcaagaaaccttaacaattgtcatatggtgaccatcacatggccactctaactcataatatctcatattgcaacattatttttgacgtgatgctataaataattaatagtccaattatgtttgtaggttaatacattacattttccagagtatctggtttcgacttttctgtttataataatgttttactttttactgaaaagtttatacagaattgctggaactggatatgtatatttgtgggatggaacaaatgagtcatttcatgttgtatgcaggatagaattagtgttaccaaacctggaactttgaatgctcaagcacgaacagaacatcaacgacgtgttcctgatgcagcatcctcattggagctgtcctctttatctgttgcacagtccatttcatcagtgccaagtgcaactctagcagaaagacgatcagcagcagcagtaaattgtagtacaggagaagtggttaagcagagttctgacgcccaggttctagctcttgtaccagttctaaagagaccaactcgcgatgggtacaattggcggaagtatggtcaaaagcaagttaaaagtcctcaaggttctcgaagttattaccgatgcactcattctgagtgttgtgccaagaagattgagtgctctgatcacactaatcgtgttatggagattatttatagaactcaacacaatcatgatccacccccaagagtaaattgcccaagggaaagcaagtctgcattattgtcttcacctaccaatggcaaaagtataatagctcatccaaggagaaattctattgagaccgtagtatcccccttaaatgaaaatttgcaagaaagtttaccaattgctgagacagcaaatcaggattcaggtgggtctgacactgacactgaaatcactattagagaggagcaccgtgacgaggctggacaaaagaagaggcaagttcacttttgtattcaattttagttattttatttttctgcttttcctcttacaaatgttcaaaaccatatgattgatcaccattctcacctatgattttcaggtcaaggaaaagtgacacaagttgtttggaatctgtttctaaacctggaaagaaacccaagcttgtggtgcatgctgcttgtgatgtaggaatctcaagtgatggctacagatggcgaaagtatggacaaaaaatagtgaagggaaatccccatccaaggtactgtattattttctgccgtacacttgataaatcgtttgattgttctgcctgccttacgctgaaattataagaactaggagggagtgatgccacattaaacacatttcttgaatcatacttgggagtttttttttctctattttctctgctttgtttccttttgttggattgtgctgatggatgagttctattcttcatgcaccctattctgctctgttaaactaagttgctcggactcttcaaaaatgttgatgggtgcatgagggatactccaacagtagtgcattttcagagaatccaacacgggtgcagcagcattttggagactccgagcaacatagttgttaaatgctatggatgagagtgtcactcatcttattcccttttctgttctgttaagacaattaggttttcttcaggtaaataattcctgctagttttctgtttcaagttagaatttcttatgattcaacatcaatattgacaactcttctcacatattacttgtttttatctacttcacgttttaactcatatcttggtcaaaagtatacttcattttgcttctttcgttctcctgttctgtcctgagttgtttcctggatgacctttaggaactactatcgctgtacatcagctggatgtcccgttcgaaagcacattgagagggttttagataccacaagtgctttaacaataacatacaagggagtacacgatcatgacatgccagtacccaaaaaacgtcatggtccaccgagtgcacctcttattgctgctactgcccctgcttccgtaaccactatgcatgctaacaaacccgaacccctacaacatcaaaaatcgaccacacaatggtccgtggacaaagaaggtgagttgactggtgagaaattggatgttggaggagaaaaagcaatggaatcggctcgaactctattgagtattggatttgaaattaagccttgctaaaattgcttagctgctctgattttatttttttctgcatttatttagttttcctccatagggctttcttgtagaagtttagaagagtacacctttttttttatagtcctccaatatatagatggtctatactcagttatgtacattattgtggatcaaaataagtaacatagaacttagaataacatattgtgatgtttgtcaatttgcatctgtttc

SEQ ID NO: 11 - DNA, 1542 bp, Solanum lycopersicum
atggatgacgaaaacgagagctccaaatcagccggactcaaaaattcaaatctagaagaagaagaagaagataaaatcagcaacaaaatcgaaaattcctccgtacacaacgacgaaaacggtgacgacgatagagtaattgacggtagcagtggagctgagagtttacgagaatcaaagacgggagctttaatttcagaaaccctagctcatcctaatgcagaatcatccgtacaaattgaaattgatggccaatccgaattcgattcagagttttctccctcttatcaactttctgaagtaccagtggaatatgaactgccctcgtttggtttctcggaaaaaatcaaggatagaattagtgttaccaaacctggaactttgaatgctcaagcacgaacagaacatcaacgacgtgttcctgatgcagcatcctcattggagctgtcctctttatctgttgcacagtccatttcatcagtgccaagtgcaactctagcagaaagacgatcagcagcagcagtaaattgtagtacaggagaagtggttaagcagagttctgacgcccaggttctagctcttgtaccagttctaaagagaccaactcgcgatgggtacaattggcggaagtatggtcaaaagcaagttaaaagtcctcaaggttctcgaagttattaccgatgcactcattctgagtgttgtgccaagaagattgagtgctctgatcacactaatcgtgttatggagattatttatagaactcaacacaatcatgatccacccccaagagtaaattgcccaagggaaagcaagtctgcattattgtcttcacctaccaatggcaaaagtataatagctcatccaaggagaaattctattgagaccgtagtatcccccttaaatgaaaatttgcaagaaagtttaccaattgctgagacagcaaatcaggattcaggtgggtctgacactgacactgaaatcactattagagaggagcaccgtgacgaggctggacaaaagaagaggtcaaggaaaagtgacacaagttgtttggaatctgtttctaaacctggaaagaaacccaagcttgtggtgcatgctgcttgtgatgtaggaatctcaagtgatggctacagatggcgaaagtatggacaaaaaatagtgaagggaaatccccatccaaggaactactatcgctgtacatcagctggatgtcccgttcgaaagcacattgagagggttttagataccacaagtgctttaacaataacatacaagggagtacacgatcatgacatgccagtacccaaaaaacgtcatggtccaccgagtgcacctcttattgctgctactgcccctgcttccgtaaccactatgcatgctaacaaacccgaacccctacaacatcaaaaatcgaccacacaatggtccgtggacaaagaaggtgagttgactggtgagaaattggatgttggaggagaaaaagcaatggaatcggctcgaactctattgagtattggatttgaaattaagccttgctaa

SEQ ID NO: 12 - DNA, 201 bp, artificial sequence
  WRKY32 RNAi encoding sequence
ctgacatgccagtacccaaaaaacgtcatggtccaccgagtgcacctcttattgctgctactgcccctgcttccgtaaccactatgcatgctaacaaacccgaacccctacaacatcaaaaatcgaccacacaatggtccgtggacaaagaaggtgagttgactggtgagaaattggatgttggaggagaaaaagcaatgg

SEQ ID NO: 13 - DNA, 2229 bp, Arabidopsis thaliana
ttttcttccggagatcagtcggtcggaaagcggctacctttttgtctgcctagagaatttgttcgtttctttcttttactctcttcagacaaaacccacgagatacagaaaaagaggacaagagagaatcgtccatggaagaagacactggtatcgacgaagctaagacatacacggtggagaagagcgagaaagtggagccggagaaggacggactgagtcaattcagagacgaggaaaaatcacttggtgcggatatggaagatttacatgatgagactgtgcgagaaaccctaggcaaggatcaggttcaaggtaacggtttattctgcgcaaaattctttattggtttttatttatttattcgagactttattttttgacgaaatgatgtttgagtttaccaggtgttcgagaaaattcctctgtggaaccaaatgttgaagatgtattagaagtgaatgtgagtttgcttcagactcttctgctattcataaactttcttaacacttacaactttgattctctcattaacattgattgtgctagaacttgtaaagtttaactcatttcagtgtcttcgatgttactcgttcagtgattatacaataacatgggaataggattaatcgtaatggttttaacctttggccaagttcaatctgtatctgtatcagtttgatctgttacattttagtgtgtctgatttcttaggcaattctgaggacaagaatcactgttatcaaggcatgacatttaactgctttttgtatcacattggcaggagactgatagcgtcaaggaaactgttgtaagtgcgattgtgccggttgatgaagtggaagagaatcgtcaggtagaaacatctccttctctggctgcatcgtcagactcattgacagtgacgccatgtctatctttggatcctgcaactgcttcaaccgcacaagatttaccactggtttcagttccaactaaacaagagcaaagatcagattcgccggtggttaacagattgtcggttactcctgttcctaggacaccggctcgtgatggttataattggagaaaatatggacagaagcaggttaagagtcccaagggctcacggagttactacaggtgtacatacactgaatgttgtgctaaaaaaattgaatgctccaatgattcaggcaatgtggtagagattgttaacaaaggtttacatactcatgaacctccccggaagactagcttctccccgagagagattagagttacaacagctatccggcctgtttcagaggatgatacagtagtagaagagctatcaattgttcctagcggttcagatccgtctgcttctactaaagaatacatctgtgagtcgcaaacactcgttgaccggaaaagacactgtgagaacgaagctgtggaggaaccagagccaaaacgaaggcaagtttgtagaattttgcatttcggtgcttactcttcactttgaaagatgaaattaatagactttcttctctctatttttcagactgaaaaaagataactcacagagttcagattctgtctccaaacctggaaagaaaaacaaattcgtagtacacgcagctggtgatgttggtatctgtggtgatggatacaggtggcgtaaatacgggcagaaaatggtgaaaggaaatcctcatccaaggtctagaaaactaaacgcatgacccatctctttatccacatatgacatcttctaatacgcatggtgattgatttgttctgtttcaaacattcaggaactactaccgatgcacttcagcgggatgtccagttcgtaaacacattgagacagcagtcgagaacacaaaagcagtaataatcacatacaaaggagtacacaaccacgacatgccggtgcctaagaaacgccatggtcctccaagctcaatgctcgtagctgcagccgctccaacatcaatgagaaccaggacagacgatcaggtgaacattccgacttcaagccagtgctcggtggggcgagaaagtgagaagcagagtaaagaagcattggacgttggtggagagaaagtgatggaatcagctaggactttgttgagcattggattcgaaatcaagcaatgctgattatatgtagtttatgagttttatagagttcatcgactcaattttcgcctccttgttcttgttatataataataataaaaaaccccatgaagattaccaact

SEQ ID NO: 14 - DNA, 1401 bp, Arabidopsis thaliana
atggaagaagacactggtatcgacgaagctaagacatacacggtggagaagagcgagaaagtggagccggagaaggacggactgagtcaattcagagacgaggaaaaatcacttggtgcggatatggaagatttacatgatgagactgtgcgagaaaccctaggcaaggatcaggttcaaggtgttcgagaaaattcctctgtggaaccaaatgttgaagatgtattagaagtgaatgagactgatagcgtcaaggaaactgttgtaagtgcgattgtgccggttgatgaagtggaagagaatcgtcaggtagaaacatctccttctctggctgcatcgtcagactcattgacagtgacgccatgtctatctttggatcctgcaactgcttcaaccgcacaagatttaccactggtttcagttccaactaaacaagagcaaagatcagattcgccggtggttaacagattgtcggttactcctgttcctaggacaccggctcgtgatggttataattggagaaaatatggacagaagcaggttaagagtcccaagggctcacggagttactacaggtgtacatacactgaatgttgtgctaaaaaaattgaatgctccaatgattcaggcaatgtggtagagattgttaacaaaggtttacatactcatgaacctccccggaagactagcttctccccgagagagattagagttacaacagctatccggcctgtttcagaggatgatacagtagtagaagagctatcaattgttcctagcggttcagatccgtctgcttctactaaagaatacatctgtgagtcgcaaacactcgttgaccggaaaagacactgtgagaacgaagctgtggaggaaccagagccaaaacgaagactgaaaaaagataactcacagagttcagattctgtctccaaacctggaaagaaaaacaaattcgtagtacacgcagctggtgatgttggtatctgtggtgatggatacaggtggcgtaaatacgggcagaaaatggtgaaaggaaatcctcatccaaggaactactaccgatgcacttcagcgggatgtccagttcgtaaacacattgagacagcagtcgagaacacaaaagcagtaataatcacatacaaaggagtacacaaccacgacatgccggtgcctaagaaacgccatggtcctccaagctcaatgctcgtagctgcagccgctccaacatcaatgagaaccaggacagacgatcaggtgaacattccgacttcaagccagtgctcggtggggcgagaaagtgagaagcagagtaaagaagcattggacgttggtggagagaaagtgatggaatcagctaggactttgttgagcattggattcgaaatcaagcaatgctga

SEQ ID NO: 15 - protein, 466 aa, Arabidopsis thaliana
MEEDTGIDEAKTYTVEKSEKVEPEKDGLSQFRDEEKSLGADMEDLHDETVRETLGKDQVQGVRENSSVEPNVEDVLEVNETDSVKETVVSAIVPVDEVEENRQVETSPSLAASSDSLTVTPCLSLDPATASTAQDLPLVSVPTKQEQRSDSPVVNRLSVTPVPRTPARDGYNWRKYGQKQVKSPKGSRSYYRCTYTECCAKKIECSNDSGNVVEIVNKGLHTHEPPRKTSFSPREIRVTTAIRPVSEDDTVVEELSIVPSGSDPSASTKEYICESQTLVDRKRHCENEAVEEPEPKRRLKKDNSQSSDSVSKPGKKNKFVVHAAGDVGICGDGYRWRKYGQKMVKGNPHPRNYYRCTSAGCPVRKHIETAVENTKAVIITYKGVHNHDMPVPKKRHGPPSSMLVAAAAPTSMRTRTDDQVNIPTSSQCSVGRESEKQSKEALDVGGEKVMESARTLLSIGFEIKQC